European Patent Application EP 4 177 264 A1, published May 10, 2023. Title: TRANSFECTED T-CELLS AND T-CELL RECEPTORS FOR USE IN IMMUNOTHERAPY AGAINST CANCERS. Applicant: Immatics Biotechnologies GmbH. The sequence listing filed with the application follows.

SEQUENCE LISTING (45 sequences)

SEQ ID NO: 1 - protein, 9 aa, Homo sapiens
KIQEILTQV

SEQ ID NO: 2 - protein, 271 aa, Homo sapiens
MKTFAGFSFLFLWLQLDCMSRGEDVEQSLFLSVREGDSSVINCTYTDSSSTYLYWYKQEPGAGLQLLTYIFSNMDMKQDQRLTVLLNKKDKHLSLRIADTQTGDSAIYFCAESKETRLMFGDGTQLVVKPNIQNPDPAVYQLRDSKSSDKSVCLFTDFDSQTNVSQSKDSDVYITDKTVLDMRSMDFKSNSAVAWSNKSDFACANAFNNSIIPEDTFFPSPESSCDVKLVEKSFETDTNLNFQNLSVIGFRILLLKVAGFNLLMTLRLWSS

SEQ ID NO: 3 - protein, 21 aa, Homo sapiens
MKTFAGFSFLFLWLQLDCMSR

SEQ ID NO: 4 - protein, 113 aa, Homo sapiens
MKTFAGFSFLFLWLQLDCMSRGEDVEQSLFLSVREGDSSVINCTYTDSSSTYLYWYKQEPGAGLQLLTYIFSNMDMKQDQRLTVLLNKKDKHLSLRIADTQTGDSAIYFCAES

SEQ ID NO: 5 - protein, 6 aa, Homo sapiens
DSSSTY

SEQ ID NO: 6 - skipped

SEQ ID NO: 7 - protein, 11 aa, Homo sapiens
CAESKETRLMF

SEQ ID NO: 8 - protein, 14 aa, Homo sapiens
RLMFGDGTQLVVKP

SEQ ID NO: 9 - protein, 141 aa, Homo sapiens
NIQNPDPAVYQLRDSKSSDKSVCLFTDFDSQTNVSQSKDSDVYITDKTVLDMRSMDFKSNSAVAWSNKSDFACANAFNNSIIPEDTFFPSPESSCDVKLVEKSFETDTNLNFQNLSVIGFRILLLKVAGFNLLMTLRLWSS

SEQ ID NO: 10 - protein, 318 aa, Homo sapiens
MLLLLLLLGPGISLLLPGSLAGSGLGAVVSQHPSWVICKSGTSVKIECRSLDFQATTMFWYRQFPKQSLMLMATSNEGSKATYEQGVEKDKFLINHASLTLSTLTVTSAHPEDSSFYICSARAGGHEQFFGPGTRLTVLEDLKNVFPPEVAVFEPSEAEISHTQKATLVCLATGFYPDHVELSWWVNGKEVHSGVSTDPQPLKEQPALNDSRYCLSSRLRVSATFWQNPRNHFRCQVQFYGLSENDEWTQDRAKPVTQIVSAEAWGRADCGFTSESYQQGVLSATILYEILLGKATLYAVLVSALVLMAMVKRKDSRG

SEQ ID NO: 11 - protein, 25 aa, Homo sapiens
MLLLLLLLGPGISLLLPGSLAGSGL

SEQ ID NO: 12 - protein, 122 aa, Homo sapiens
MLLLLLLLGPGISLLLPGSLAGSGLGAVVSQHPSWVICKSGTSVKIECRSLDFQATTMFWYRQFPKQSLMLMATSNEGSKATYEQGVEKDKFLINHASLTLSTLTVTSAHPEDSSFYICSAR

SEQ ID NO: 13 - protein, 6 aa, Homo sapiens
DFQATT

SEQ ID NO: 14 - protein, 7 aa, Homo sapiens
SNEGSKA

SEQ ID NO: 15 - protein, 12 aa, Homo sapiens
CSARAGGHEQFF

SEQ ID NO: 16 - protein, 13 aa, Homo sapiens
EQFFGPGTRLTVL

SEQ ID NO: 17 - protein, 179 aa, Homo sapiens
EDLKNVFPPEVAVFEPSEAEISHTQKATLVCLATGFYPDHVELSWWVNGKEVHSGVSTDPQPLKEQPALNDSRYCLSSRLRVSATFWQNPRNHFRCQVQFYGLSENDEWTQDRAKPVTQIVSAEAWGRADCGFTSESYQQGVLSATILYEILLGKATLYAVLVSALVLMAMVKRKDSRG

SEQ ID NO: 18 - protein, 20 aa, Homo sapiens
VIGFRILLLKVAGFNLLMTL

SEQ ID NO: 19 - protein, 23 aa, Homo sapiens
TILYEILLGKATLYAVLVSALVL

SEQ ID NO: 20 - protein, 274 aa, Homo sapiens
METLLGLLILWLQLQWVSSKQEVTQIPAALSVPEGENLVLNCSFTDSAIYNLQWFRQDPGKGLTSLLLIQSSQREQTSGRLNASLDKSSGRSTLYIAASQPGDSATYLCAVRPTSGGSYIPTFGRGTSLIVHPYIQNPDPAVYQLRDSKSSDKSVCLFTDFDSQTNVSQSKDSDVYITDKTVLDMRSMDFKSNSAVAWSNKSDFACANAFNNSIIPEDTFFPSPESSCDVKLVEKSFETDTNLNFQNLSVIGFRILLLKVAGFNLLMTLRLWSS

SEQ ID NO: 21 - protein, 311 aa, Homo sapiens
MSIGLLCCAALSLLWAGPVNAGVTQTPKFQVLKTGQSMTLQCAQDMNHEYMSWYRQDPGMGLRLIHYSVGAGITDQGEVPNGYNVSRSTTEDFPLRLLSAAPSQTSVYFCASSYVGNTGELFFGEGSRLTVLEDLKNVFPPEVAVFEPSEAEISHTQKATLVCLATGFYPDHVELSWWVNGKEVHSGVSTDPQPLKEQPALNDSRYCLSSRLRVSATFWQNPRNHFRCQVQFYGLSENDEWTQDRAKPVTQIVSAEAWGRADCGFTSESYQQGVLSATILYEILLGKATLYAVLVSALVLMAMVKRKDSRG

SEQ ID NO: 22 - DNA, 36 bp, Homo sapiens
  source 1..36: mol_type = other DNA
ggaattccatatgagtcaacaaggagaagaagatcc

SEQ ID NO: 23 - DNA, 36 bp, Homo sapiens
  source 1..36: mol_type = other DNA
ttgtcagtcgacttagagtctctcagctggtacacg

SEQ ID NO: 24 - DNA, 36 bp, Homo sapiens
  source 1..36: mol_type = other DNA
tctctcatatggatggtggaattactcaatccccaa

SEQ ID NO: 25 - DNA, 32 bp, Homo sapiens
  source 1..32: mol_type = other DNA
tagaaaccggtggccaggcacaccagtgtggc

SEQ ID NO: 26-36 - skipped (11 entries)

SEQ ID NO: 37 - protein, 9 aa, Homo sapiens
AIQEILTQV

SEQ ID NO: 38 - protein, 9 aa, Homo sapiens
KAQEILTQV

SEQ ID NO: 39 - protein, 9 aa, Homo sapiens
KIAEILTQV

SEQ ID NO: 40 - protein, 9 aa, Homo sapiens
KIQAILTQV

SEQ ID NO: 41 - protein, 9 aa, Homo sapiens
KIQEALTQV

SEQ ID NO: 42 - protein, 9 aa, Homo sapiens
KIQEIATQV

SEQ ID NO: 43 - protein, 9 aa, Homo sapiens
KIQEILAQV

SEQ ID NO: 44 - protein, 9 aa, Homo sapiens
KIQEILTAV

SEQ ID NO: 45 - protein, 9 aa, Homo sapiens
KIQEILTQA